European Patent Application EP 4 116 431 A1, published January 11, 2023. Title: DETECTION OF ATYPICAL PNEUMONIA. Applicant: QUEST DIAGNOSTICS INVESTMENTS INCORPORATED. Application New divisional application based on EP19161780.2. The sequence listing filed with the application follows.

SEQUENCE LISTING (49 sequences)

SEQ ID NO: 1 - DNA, 5146 bp, Mycoplasma pneumoniae
gctttaaagtatggtggcgggggtcatattcaggccagcggtgcagttcttaaaagcaagcgcgacataattcgtgtagttcaagattgccaaaagcaaattgctgtataatttttaacaactatgcaccaaaccaaaaaaactgccttgtccaagtccacttggattctcatcctcaccgccaccgcctccctcgcgacgggactcaccgtagtgggacacttcacaagtaccaccacgacgctcaagcgccagcaatttagctacacccgccctgacgaggtcgcgctgcgccacaccaatgccatcaacccgcgcttaaccccgtgaacgtatcgtaacacgagcttttcctccctccccctcacgggtgaaaatcccggggcgtgggccttagtgcgcgacaacagcgctaagggcatcactgccggcagtggcagtcaacaaaccacgtatgatcccacccgaaccgaagcggctttgaccgcatcaaccacctttgcgttacgccggtatgacctcgccgggcgcgccttatacgacctcgatttttcgaagttaaacccgcaaacgcccacgcgcgaccaaaccgggcagatcacctttaacccctttggcggctttggtttgagtggggctgcaccccaacagtgaaacgaggtcaaaaacaaggtccccgtcgaggtggcgcaagacccctccaatccttatcggtttgccgttttactcgtgccgcgtagcgtggtgtactatgagcagttgcagcgggggttagcgctccctaaccaagggagttcgtcaggctcagacagcactaaccaaacaggcgcaatgtttggcttgaaggtgaaggatgcaaccgtggatagttcgaagcaatcaacggaaagcttaaagggcgaagaatcgagttccagttccaccacatcttccacctccaccacccaacgtgggggttcgtcaaatgaaaacaaagtcaaggcgttgcaggtggcggtgaaaaagaaatccgggagtcagggcaactccggtgaccaaggcaccgaacaggtggaacttgaatctaatgatttagccaacgccccgattaaacggggctccaataacaaccagcaagtccaactcaaggcggacgattttggtactgccccttccagttcgggatcaggcacccaagatggcacccccaccccctgaacgccgtggttaacgactgagcaaattcacaacgaccccgccaaattcgccgcctcgatcctgattctgtacgatgcgccttatgcgcgcaaccgtaccgccattgaccgcgttgatcacttggatcccaaggccatgaccgcgaactatccgcccagttgaagaacgcccaagtgaaaccaccacggtttgtgggactgaaaggcgcgcgatgttttgctccaaaccaccgggttcttcaacccgcgccgccaccccgagtggtttgatggcgggcagacggtcgcggataacgaaaagaccgggtttgatgtggataactctgaaaacaccaagcagggctttcaaaaggaagctgactccgacaagtcggccccgatcgccctcccgtttgaagcgtacttcgccaacattggcaacctcacctggttcgggcaagcgcttttggtgtttggtggcaatggccatgttaccaagtcggcccacaccgcgcctttgagtataggtgtctttagggtgcgctataatgcaactggtaccagtgctactgtaactggttgaccatatgccttactgttctcaggcatggtcaacaaacaaactgacgggttaaagaatctaccctttaacaataaccgctggtttgaatatgtaccacggatggcagttgctggcgctaagttcgttggtagggaactcgttttagcgggtaccattaccatgggtgataccgctaccgtacctcgcttactgtacgatgaacttgaaagcaacctgaacttagtagcgcaaggccaaggtcttttacgcgaagacttgcaactcttcacaccctacggatgagccaatcgtccggatttaccaatcggggcttgaagtagtagtagtagtagtagtcacaacgcaccctactacttccacaataaccccgattgacaagaccgtccaatccaaagtgtggttgatgcctttattaagccctgagaggacaagaacggtaaggatgatgccaaatacatctacccttaccgttacagtggcatgtgagcttgacaggtatacaactggtccaataagctcactgaccaaccattaagtgctgactttgtcaatgagaatgcttaccaaccaaactccttgtttgctgctattctcaatccggaattgttagcagctcttcccgacaaggttaaatacggtaaggaaaacgagtttgctgctaacgagtacgagcgctttaaccagaagttaacggtagctcctacccaaggaacaaactgatcccacttctcccccacgctttcccgtttctccaccgggttcaaccttgtggggtcggtgctcgaccaggtgttggattatgtgccctggattgggaatgggtacaggtatggcaataaccaccggggcgtggatgatataaccgcgcctcaaaccagcgcggggtcgtccagcggaattagtacgaacacaagtggttcgcgttcctctctcccgacgttttccaacatcggcgtcggcctcaaagcgaatgtccaagccaccctcgggggcagtcagacgatgattacaggcggttcgcctcgaagaaccctcgaccaagccaacctccagctctgaacgggggcggggtgaaggaatgataaggcttcaagtggacaaagtgacgaccacaccaagttcacgagcgctacggggatgggccagcaggaacaatcaggtacctccgcggggaatcccgactcgttaaagcaggataagattagtaagagtggggatagtttaaccacgcaggacggcaatgcgatggaacaacaagaggccaccaactacaccaacctcccccccaacctcacccccaccgctgattgaccgaacgcgctgtcattcaccaacaagaacaacgcgcagcgcgcccagctgttcctgcgcggcctgttgggcagcatcccggtgttggttaataagtccggccaagatgataacagtaagtttaaggcggaggaccaaaaatggtcctacaccgacttacagtcggaccaaaccaaactgaacctccccgcttacggtgaggtgaatgggttgttgaatccggcgttggtggaaacctattttgggaacacgcgagcgagtggttcggggtccaacacgaccagttcacccggtatcggttttaaaattcccgaacaaagtggcacaaacacaacgtcgaaggctgtgctgatcacccccgggttggcttgaacgccgcaagacgttggtaacctcgttgtcagtggcaccagcttcagcttccagctcggcgggtggttagttacgttcacggactttatcaaaccccgcgctggttacctcgggctccagttaacgggcttggatgcaagtgatgcgacgcagcgcgctctcatttgggccccccggccctgagcggcctttcgtggcagttgggtcaaccggttgggccgcgtggagagtgtgtgggatttgaagggggtgtgggcggatcaagctcagtccgactcgcaaggatctaccaccaccgcaacaagggacgccttaccggagcacccgaatgctttggcctttcaggtgagtgtggtggaagcgagtgcttacaagccaaacacgagctccggccaaacccaatccactaacagttccccctacctgcacttggtgaagcctaagaaagttatccaatccgacaagttagacgacgatcttaaaaacctgttggaccccaaccaggttcgcaccaagctgcgccaaagctttggtacagaccattccacccagccccagccccaatcgctcaaaacaacgacaccgatatttgggacgagtagtggtaacctcagtagtgtgcttagtggtgggggtgctggagggggttcttcaggctcaggtcaatctggcgtggatctctcccccgttgaaaaagtgagtgggtggcttgtggggcagttaccaagcacgagtgacggaaacacctcctccaccaacaacctcgcgcctaatactaatacggggaatgatgtggtgggggttggtcgactttctgaaagcaacgccgcaaagatgaacgacgatgttgatggtattgtacgcaccccactcgctgaactgttagatggggaaggacaaacagctgacactggtccacaaagcgtgaagttcaagtctcctgaccaaattgacttcaaccgcttgtttacccacccagtcaccgatctgtttgatccggtaactatgttggtgtatgaccagtacataccgctgtttattgatatcccagcaagtgtgaaccctaaaatggttcgtttaaaggtcttgagctttgacaccaacgaacagagcttaggtctccgcttagagttctttaaacctgatcaagatacccaaccaaacaacaacgttcaggtcaatccgaataacggtgacttcttaccactgttaacggcctccagtcaaggtccccaaaccttgtttagtccgtttaaccagtgacctgattacgtgttgccgttagcgatcactgtacctattgttgtgattgtgctcagtgttaccttaggacttgccattggaatcccaatgcacaagaacaaacaggccttgaaggctgggtttgcgctatcaaaccaaaaggttgatgtgttgaccaaagcggttggtagtgtctttaaggaaatcattaaccgcacaggtatcagtcaagcgccaaaacgcttgaaacaaaccagtgcggctaaaccaggagcaccccgcccaccagtaccaccaaagccaggggctcctaagccaccagtgcaaccacctaaaaaacccgcttagtatttatgaaatcgaagctaaagttaaaacgttatttactgtttttaccacttttaccgctaggacgttgtcactagccaacacctacctcctccaagaccacaacaccctcacc

SEQ ID NO: 2 - DNA, 200 bp, Mycoplasma pneumoniae
ccggggcgtggatgatataaccgcgcctcaaaccagcgcggggtcgtccagcggaattagtacgaacacaagtggttcgcgttcctctctcccgacgttttccaacatcggcgtcggcctcaaagcgaatgtccaagccaccctcgggggcagtcagacgatgattacaggcggttcgcctcgaagaaccctcgaccaag

SEQ ID NO: 3 - DNA, 20 bp, Mycoplasma pneumoniae
ggttcgcgttcctctctccc

SEQ ID NO: 4 - DNA, 23 bp, Mycoplasma pneumoniae
cagcggaattagtacgaacacaa

SEQ ID NO: 5 - DNA, 18 bp, Mycoplasma pneumoniae
cgaatgtccaagccaccc

SEQ ID NO: 6 - DNA, 1482 bp, Chlamydia pneumoniae
atgcttaatcatgctaaaaagcacgctaaaccctatgttcttattttcttttcgacaaaagacaagttaagttactgtgatattattttcaacaactgctctgggaaacctatgaatctagattcgaaacattttgatataaatagtgcaaatttcctggaagagtttgcaaaatttataagcttcccctcgatatctgcggatagtgatcatcttcaggattgtgaaaattgtgcacattttttagtagatcatgtgaataagattttcgatgtagagctctgggaaacgcctgggcatccccctatcatctatgcatcctataaaagcgaagatcctcttagccctactcttatgctctataaccactatgatgtgcagccagcacagctatctgatggttggaagggagatccctttatccttagagaagagaatggcaatctctatgcccgaggagcctctgataacaaaggacaatgtttttacaccttaaaggcattacagcactattacgaatctcaaggaaacttccctctaaatattatttggttaattgagggtgaagaagagagtgggagtctcgcattatttacttggttagaaaagaaaaaagaagctttacgcgcggactatcttctgatcgtagatgggggtttcctttctgaaaaacacccctacgtaagcattggagctcggggtattgtttccatgaaaatctcccttgaagaggggaacaaggacatgcactcaggagttttaggaggaattgcctacaatacgaatcgtgctttatcagaaattctgagctctctgcatcaccctgacaattctatagctattgaaggattttatgatgatcttgctctcccctcggatagcgatcgtcctgatcttccgaagtcggatacccttcgggaatgcgaagaaaacttagggtttcgacctcagggttacgaagcttcttatagccctgaagaatctgcgttacgtcctactgtagaaatcaatggaatttctggaggttatacgggaccaggatttaagactgtgatcccctatagagccactgcctacctctcctgccgacttgttcctaatcaagatcctgataaagctgctcaccaagttatccatcacttgaaacaacaagtcccttcttcgttaaagttctcttatgaaattcttccaggaggatctcgaggttggagaagttctgcgaacctcccaatagtcaaagtgcttcaagagatctatagtgacctctacaatgaagaatgcctgagattagtgatgcctgctacgatcccgataggtcccctattaggggaagcagcacaaacctcacctatcatttgtgggacttcgtatcttagtgatgatattcacgctgcagaagagcatttctcgatggaccaacttaaaaagggattcctttctatttgtcagcttcttgataagcttcctaaaataaaagagtga

SEQ ID NO: 7 - DNA, 250 bp, Chlamydia pneumoniae
attacagcactattacgaatctcaaggaaacttccctctaaatattatttggttaattgagggtgaagaagagagtgggagtctcgcattatttacttggttagaaaagaaaaaagaagctttacgcgcggactatcttctgatcgtagatgggggtttcctttctgaaaaacacccctacgtaagcattggagctcggggtattgtttccatgaaaatctcccttgaagaggggaacaaggacatgcac

SEQ ID NO: 8 - DNA, 21 bp, Chlamydia pneumoniae
cgcggactatcttctgatcgt

SEQ ID NO: 9 - DNA, 25 bp, Chlamydia pneumoniae
ggagtctcgcattatttacttggtt

SEQ ID NO: 10 - DNA, 18 bp, Chlamydia pneumoniae
taagcattggagctcggg

SEQ ID NO: 11 - DNA, 1189 bp, Legionella pneumophila
gttgatgatatgggggctgataaattgattcaggcgaaatgtgtaaaaaataatgaacagattaatttgagaatttcagcagagcagatggtctcaaacaggcaattacatgtagagctacccaaattgaaattgcatgtatttgatgagagaacaggaaaacgtgtgggagagtggcgtggctaaagaaaaaaataaattaaaaccgattgatgctcctatctatagttattggcaagcgctgtatatgtctttttattcaaagaggctttttgttgatgtaggaaaacattggcgtggaattggtttgatttatctattattggttattgctatttgttcaataccgttttctataagaattgcttctgattttaataaaacgtttaatcagcaaatcattgaacctttgctgcagctgccaactgtttatgtacaaaaaggtaatgttatttttgataaaccaatgccctatttaatcagaaatgataaaaatcaagtggtaataattatagacacaacaggcaaagtggtagatttcacagaggagtatccttaccttaatattctgattaagaaaaatagtattaatttcttattgccaacaccagaattattgggtagcagcccagtaaatgaacagaaaggagttcctattgttcagccattagataaagacatgaatatggtatttgatggcaaaaaaattattcaggataatgcgattaatggtttgaaatatgcctctcaattgatgatatatccaatagtggttgctattttatattcgattatggtgactgttttattggtcattgcgtttttaggacaagtattttccaaaatctttttttcgttcactatatcctttaaaaaatccagccgtctgttaatggtcgcatcaacgccaatgttagtagttttggtaaccatgttatcacttcattttatttttccaggatttggagtgattttgttgatattattggcagcctattacagttacggtgtctatggtctccgagatgaaagcaggaaaatggtgctcaaatgagagagttaatccattttgctcatggcaatggatttccatcattatgttacaaacagttactagagcagctggaggctcgttttgactgttgttttatagataaaattggacatgatcctcattatcctgtcggag

SEQ ID NO: 12 - DNA, 170 bp, Legionella pneumophila
gtctcaaacaggcaattacatgtagagctacccaaattgaaattgcatgtatttgatgagagaacaggaaaacgtgtgggagagtggcgtggctaaagaaaaaaataaattaaaaccgattgatgctcctatctatagttattggcaagcgctgtatatgtctttttatt

SEQ ID NO: 13 - DNA, 18 bp, Legionella pneumophila
gtgggagagtggcgtggc

SEQ ID NO: 14 - DNA, 25 bp, Legionella pneumophila
gcatgtatttgatgagagaacagga

SEQ ID NO: 15 - DNA, 27 bp, Legionella pneumophila
tgatgctcctatctatagttattggca

SEQ ID NO: 16 - DNA, 27 bp, Legionella pneumophila
atgctcctatctatagttattggcaag

SEQ ID NO: 17 - DNA, 21 bp, Legionella pneumophila
ttggcaagcgctgtatatgtc

SEQ ID NO: 18 - DNA, 27 bp, Artificial Sequence
  Description of Artificial Sequence: Synthetic primer
agcgggagagaggaacgcgaacccgct

SEQ ID NO: 19 - DNA, 18 bp, Artificial Sequence
  Description of Artificial Sequence: Synthetic primer
gggtggcttggacattcg

SEQ ID NO: 20 - DNA, 30 bp, Artificial Sequence
  Description of Artificial Sequence: Synthetic primer
ccgacgatcagaagatagtccgcgcgtcgg

SEQ ID NO: 21 - DNA, 18 bp, Artificial Sequence
  Description of Artificial Sequence: Synthetic primer
cccgagctccaatgctta

SEQ ID NO: 22 - DNA, 27 bp, Artificial Sequence
  Description of Artificial Sequence: Synthetic primer
agcgccgtgggagagtggcgtggcgct

SEQ ID NO: 23 - DNA, 25 bp, Artificial Sequence
  Description of Artificial Sequence: Synthetic primer
gcatgtatttgatsagagaacagga

SEQ ID NO: 24 - DNA, 27 bp, Artificial Sequence
  Description of Artificial Sequence: Synthetic primer
agcgccacgccactctcccacggcgct

SEQ ID NO: 25 - DNA, 27 bp, Artificial Sequence
  Description of Artificial Sequence: Synthetic primer
cttgccaataactatagataggagcat

SEQ ID NO: 26 - DNA, 77 bp, Artificial Sequence
  Description of Artificial Sequence: Synthetic oligonucleotide
aattcgccctttgtttcgacctagcttgccagttcgcagaatttgttgctcgtcagtcgtcggcggttttaagggcg

SEQ ID NO: 27 - DNA, 77 bp, Artificial Sequence
  Description of Artificial Sequence: Synthetic oligonucleotide
aattcgcccttaaaaccgccgacgactgacgagcaacaaattctgcgaactggcaagctaggtcgaaacaaagggcg

SEQ ID NO: 28 - DNA, 23 bp, Artificial Sequence
  Description of Artificial Sequence: Synthetic primer
gttttcccagtcacgacgttgta

SEQ ID NO: 29 - DNA, 22 bp, Artificial Sequence
  Description of Artificial Sequence: Synthetic primer
cactttatgcttccggctcgta

SEQ ID NO: 30 - DNA, 258 bp, Artificial Sequence
  Description of Artificial Sequence: Synthetic polynucleotide
gttttcccagtcacgacgttgtaaaacgacggccagtgaattcgcccttaaaaccgccgacgactgacgagcaacaaattctgcgaactggcaagctaggtcgaaacaaagggcggattcgagctcggtacccggggatcctctagagtcgacctgcaggcatgcaagcttggcgtaatcatggtcatagctgtttcctgtgtgaaattgttatccgctcacaattccacacaacatacgagccggaagcataaagtg

SEQ ID NO: 31 - DNA, 34 bp, Artificial Sequence
  Description of Artificial Sequence: Synthetic primer
accagggaattcagcggaattagtacgaacacaa

SEQ ID NO: 32 - DNA, 30 bp, Artificial Sequence
  Description of Artificial Sequence: Synthetic primer
tgacttggatccgggtggcttggacattcg

SEQ ID NO: 33 - DNA, 36 bp, Artificial Sequence
  Description of Artificial Sequence: Synthetic primer
tgaagaggatccggagtctcgcattatttacttggt

SEQ ID NO: 34 - DNA, 30 bp, Artificial Sequence
  Description of Artificial Sequence: Synthetic primer
gaaacactgcagcccgagctccaatgctta

SEQ ID NO: 35 - DNA, 36 bp, Artificial Sequence
  Description of Artificial Sequence: Synthetic primer
caaatctgcaggcatgtatttgatgagagaacagga

SEQ ID NO: 36 - DNA, 32 bp, Artificial Sequence
  Description of Artificial Sequence: Synthetic primer
cagataagcttgacatatacagcgcttgccaa

SEQ ID NO: 37 - DNA, 23 bp, Artificial Sequence
  Description of Artificial Sequence: Synthetic primer
gttttcccagtcacgacgttgta

SEQ ID NO: 38 - DNA, 22 bp, Artificial Sequence
  Description of Artificial Sequence: Synthetic primer
cactttatgcttccggctcgta

SEQ ID NO: 39 - DNA, 483 bp, Artificial Sequence
  Description of Artificial Sequence: Synthetic polynucleotide
gttttcccagtcacgacgttgtaaaacgacggccagtgaattcagcggaattagtacgaacacaagtggttcgcgttcctctctcccgacgttttccaacatcggcgtcggcctcaaagcgaatgtccaagccacccggatccggagtctcgcattatttacttggttagaaaagaaaaaagaagctttacgcgcggactatcttctgatcgtagatgggggtttcctttctgaaaaacacccctacgtaagcattggagctcgggctgcaggcatgtatttgatgagagaacaggaaaacgtgtgggagagtggcgtggctaaagaaaaaaataaattaaaaccgattgatgctcctatctatagttattggcaagcgctgtatatgtcaagcttggcgtaatcatggtcatagctgtttcctgtgtgaaattgttatccgctcacaattccacacaacatacgagccggaagcataaagtg

SEQ ID NO: 40 - DNA, 24 bp, Artificial Sequence
  Description of Artificial Sequence: Synthetic primer
agcgtgcgaactggcaagcacgct

SEQ ID NO: 41 - DNA, 18 bp, Artificial Sequence
  Description of Artificial Sequence: Synthetic primer
ccgacgactgacgagcaa

SEQ ID NO: 42 - DNA, 21 bp, Artificial Sequence
  Description of Artificial Sequence: Synthetic primer
tggtgactgcagctgttatgg

SEQ ID NO: 43 - DNA, 22 bp, Artificial Sequence
  Description of Artificial Sequence: Synthetic primer
cggcaccaatgctataagacaa

SEQ ID NO: 44 - DNA, 23 bp, Artificial Sequence
  Description of Artificial Sequence: Synthetic probe
atggctgcaaccgatgccacatc

SEQ ID NO: 45 - DNA, 23 bp, Artificial Sequence
  Description of Artificial Sequence: Synthetic primer
cagcggaattagtacgaacacaa

SEQ ID NO: 46 - DNA, 24 bp, Artificial Sequence
  Description of Artificial Sequence: Synthetic primer
ggagtctcgcattatttacttggt

SEQ ID NO: 47 - DNA, 27 bp, Artificial Sequence
  Description of Artificial Sequence: Synthetic primer
tgccaataactatagataggagcatca

SEQ ID NO: 48 - DNA, 25 bp, Artificial Sequence
  Description of Artificial Sequence: Synthetic primer
gcatgtatttgatgagagaacagga

SEQ ID NO: 49 - DNA, 22 bp, Artificial Sequence
  Description of Artificial Sequence: Synthetic primer
attcgccctttgtttcgaccta